European Patent Application EP 4 502 158 A1, published February 5, 2025. Title: COCHLEAR AND/OR VESTIBULAR CELL-SPECIFIC PROMOTER AND USE THEREOF. Applicant: Shanghai Emaygene Technology Co.,Ltd. Application AM 18850555, filed March 15, 2023. The sequence listing filed with the application follows.

SEQUENCE LISTING (38 sequences)

SEQ ID NO: 1 - DNA, 1968 bp, STRC promoter sequence
  source 1..1968: mol_type = other DNA
acaatatcagttcttgaggccaagtagctgctgttggcaaggattaactactgtcatgttttgaccagggtctgcaccaccctagggaacttcaagttccctatgaggctattgtcaagaccaatagccacttgactcaacttgtggaaatagtgttcacaaagtttccatattaggaacttaccaatcatcttgtaaaaacctacaccaaagtgtctgggcagagaacctaggctctggctatggttacaatagagggcatatgtatattttgatttttttttttttgagatggtttcactatgtaaccctggctagcccgaacttgttatatagacaaggctggactcagactcacagagatcatcctgcctctgcctcttaagtgctgggattaaaagcctgtgccaccattcccagcccaacacatttgtttgtttgcttgagaaagggtttctctgtgtagcccaggatgtcctgaaactcactctgtagactaggctggtctcaaactcagtgagccacctgcctttacctcctgagtgctgctgttaaaggcatgtgccaccaccatctagcttgattttttaattaattttttaaaaaacgtgtagtatacatgtaatggtgtgttcctttaatcccagcactcaggctgacagaggcaggcagagctctgtgagtttaaggccagcctaatctacatagagaattccaccgcagccagggctacctggggagaccctatctcaatgatacgatgatgatggatgacttgactgaatggatatctgtgcaccatgtgcatacctggttccctcagagaccagaagaggaggtcagatgccctgaactggaattagagatggttgtgagcagccatatgaatgctgggaatcaaacccaggtcctctgggtttggaagagcagcagtcactgttctaatctgctgagccatccctctagacctgctcataaggtttttttatgcaagaagagatgaccagtctctggacagaccagcttatattgaatgaaatctttctaacccatgaataggattccatgtgtagagagttttaacttgagaaagaaaaagaaactgcaatgtttacatggcctaatcaagtaacagctctctgagtctctctccttacctgttaattgaagggtttacctatgtggtttgtgaagtcctgtctactccttaatattgcaggattccaaggatttatttttatgtgtgtatgtgtgttgtatctgtgtaggcatgggcaggttaagtgcagacgcccacagaggcaagagacatcagattcccctggagctggagttacaggcagttctgaaccacccaattcaggtgcatgtaactcaactcaggtcatctgcaaaggcagcatacactctcagctgctgagccatctcttcagcaccaatactgtgggactctggatagtgtgtctaaggtaacaactctcctcttcctaaatagtctacccttgaaacatctatcttaatatcttctcgctgcccactgctggctgccagaccatttctcaaattcttcaaatctcagttgtctctcaaactccttttgtactttctttgtttgatcacatttttctgtagacccccagattatatttttagtctgccttcttctctctggctcttaactcatgccgtctccttgggtaatactctgagggccccgagatcccctgtcattggtccctctaacagaagtacacccttctcccaaagccagaggatcaggtgttcagtggctccggtgacaggtgtgatgtcaggttacagatactgtttcctgagagaccacacgacagtgtcagaggaaccccagcctgcccacaatgccccgtcttcacctggctatcccttcatggtgagcatagccagaactcacctctaggcccagtgtgcacctggaaatggtacctcgac

SEQ ID NO: 2 - DNA, 1092 bp, STRC mini promoter
  source 1..1092: mol_type = other DNA
gtgctcgagagcagccatatgaatgctgggaatcaaacccaggtcctctgggtttggaagagcagcagtcactgttctaatctgctgagccatccctctagacctgctcataaggtttttttatgcaagaagagatgaccagtctctggacagaccagcttatattgaatgaaatctttctaacccatgaataggattccatgtgtagagagttttaacttgagaaagaaaaagaaactgcaatgtttacatggcctaatcaagtaacagctctctgagtctctctccttacctgttaattgaagggtttacctatgtggtttgtgaagtcctgtctactccttaatattgcaggattccaaggatttatttttatgtgtgtatgtgtgttgtatctgtgtaggcatgggcaggttaagtgcagacgcccacagaggcaagagacatcagattcccctggagctggagttacaggcagttctgaaccacccaattcaggtgcatgtaactcaactcaggtcatctgcaaaggcagcatacactctcagctgctgagccatctcttcagcaccaatactgtgggactctggatagtgtgtctaaggtaacaactctcctcttcctaaatagtctacccttgaaacatctatcttaatatcttctcgctgcccactgctggctgccagaccatttctcaaattcttcaaatctcagttgtctctcaaactccttttgtactttctttgtttgatcacatttttctgtagacccccagattatatttttagtctgccttcttctctctggctcttaactcatgccgtctccttgggtaatactctgagggccccgagatcccctgtcattggtccctctaacagaagtacacccttctcccaaagccagaggatcaggtgttcagtggctccggtgacaggtgtgatgtcaggttacagatactgtttcctgagagaccacacgacagtgtcagaggaaccccagcctgcccacaatgccccgtcttcacctggctatcccttcatggtgagcatagccagaactcacctctaggcccagtgtgcacctggaaat

SEQ ID NO: 3 - DNA, 47 bp, upstream primer
  source 1..47: mol_type = other DNA
ctattaccatggtgctcgagacaatatcagttcttgaggccaagtag

SEQ ID NO: 4 - DNA, 41 bp, downstream primer
  source 1..41: mol_type = other DNA
gcccagtgtgcacctggaaatggtacctcgacggtaagtcc

SEQ ID NO: 5 - DNA, 409 bp, CMV enhancer
  source 1..409: mol_type = other DNA
gttcctgcggccgcacgcgtgacattgattattgactagttattaatagtaatcaattacggggtcattagttcatagcccatatatggagttccgcgttacataacttacggtaaatggcccgcctggctgaccgcccaacgacccccgcccattgacgtcaataatgacgtatgttcccatagtaacgccaatagggactttccattgacgtcaatgggtggactatttacggtaaactgcccacttggcagtacatcaagtgtatcatatgccaagtacgccccctattgacgtcaatgacggtaaatggcccgcctggcattatgcccagtacatgaccttatgggactttcctacttggcagtacatctacgtattagtcatcgctattaccatggtgctcgag

SEQ ID NO: 6 - DNA, 812 bp, promoter Slc26a5
  source 1..812: mol_type = other DNA
cacgcgttctcgattctagaccatagcaaggagaggaaatgaaagtcaaaccagtttgcaacagaaagaaacttaagggtaaagaattcctaggtaaggctgataccgtaagtgtactgctggacagcgctctggtctgttacgtaacaccgggagccccattctgtcgcacagaactgcctttttctctccttaactactctgaaactagacagaattacatggtcctcattaatttatgagtgataccaaaaggatcggctcaatccgggcttcagtgtatccaggcacaggactgtgctgtgcctcctctctactcccacaatgctttgctgcgttctcagcttcccatctcctttgatgggtgaaactctcgcctatctgtgttgatcagctgttctgaaaggccccaggagatgatagcatctcttctctgggtatccatgccagtgtttaatagcctcttgaaactgccgagaagtgctcagcaattgtgtggtggggaaggacggtgtcagcaaggaataaagatgatctctcgcctcgacggtagctgaaatgtgagtttctgtgtccaggctcagataaaaagtgatcctcacacctttctcaagtagccagagacgattgaatttctggaccagggcaggaaaacaagagcatgttgctaaccttgcttagtgctggggacctgatcttcttgccattacattgtcatttctatcattctcattcttgaaaaattatcctttgatttagagataacttatgacaatgtgactctttatcttcctttctttctctctttcttt

SEQ ID NO: 7 - DNA, 542 bp, SHH mini promoter
  source 1..542: mol_type = other DNA
ctttctttctctctttctttcttttttaaactggaagccttcaggtgaaaataaagccacagcagccagaggggggagaaatgtagtctttctcagggttaacatcagaagacaagcttgtgcggcttggccaatcagatgcgcccctgccagctataatatagtgcgaaaggcagcctgtctcacaagctctccagccttgctaccatttaaaatcaggctctttttgtcttttaattgctgtctcgagacccaactccgatgtgttccgttaccagcgaccggcagcctgccatcgcagccccagtctgggtggggatcggagacaagtcccctgcagcagcggcaggcaaggttatataggaagagaaagagccaggcagcgccagagggaacgaacgagccgagcgaggaagggagagccgagcgcaaggaggagcgcacacgcacacacccgcgcgtacccgctcgcgcacagacagcgcggggacagctcacaagtcctcaggttccgcggacgaggctagcgaattcgccaccat

SEQ ID NO: 8 - DNA, 20 bp, upstream homologous arm of Slc26a5
  source 1..20: mol_type = other DNA
cacgcgttctcgattctaga

SEQ ID NO: 9 - DNA, 20 bp, downstream homologous arm of Slc26a5
  source 1..20: mol_type = other DNA
ctttctttctctctttcttt

SEQ ID NO: 10 - DNA, 20 bp, downstream homologous arm of SHH mini promoter
  source 1..20: mol_type = other DNA
gctagcgaattcgccaccat

SEQ ID NO: 11 - DNA, 1968 bp, otof promoter
  source 1..1968: mol_type = other DNA
cacgcgttctcgattctagagtactacagcccacagaagagcagtttatccttgtctaccatgtgtgtcccagggatcaaactccagtcgccaggctgagccgtaggagcccttacctgctgagccatcccaccagcccaaagcctgaagactctcttagacaggcccctgagcttccaagccctgtcagtattagttggacatcttgccatgtcttgaacactagatgccctgtgaagatctcgagtgaaaagcatcagtgggggagatccatgtagcaaccccaggccagtgatacctggatcaggagccactgaaagggggtcccaaagtccacctgagtgagggtgcagagtcacccctggggataagccgctgagaccaggaggcagggacaagatgggggacccctaccaagagtgagccgcaaaagcaacggcttagaatccagcccccagcactcctttccctacaagcccttcccgaaagagcagacttctgctgttccttggatatccctctacagatatccctctgctacctctagccactgactagagcagggagcaagatggttgtcctctcactgaaaactactcatcaatagtgtcgcctcctccagttctttgtctccagcctgggatgggtaggttggtgccctgactcttacaagtttcctacctagcacagtagcccctgtgacctctcattagggcttccctagtcacagtctctcatttcaggaccagctgcctgaaattcaaaactatgacccaagaacagagcattagagcctagcatcccaagggcacaaacagtgcaggaccaggcatcaatgcattgtcacttctgatgctcctatataataggggccagtccttggggacctccttcaaactgccttatagaagctgctgctctccagactgtgtgtgtgtgtgtgtgtgtgtgtgtgtgtgtgtgtgtgtgtgtgtgtgtgtatgtgtgtgtgtgtgtagtgtgtagatatacagatgtgtttatgtttatgtgtggaagcctagggtcaacttcagttgtcttccttatttatttatctgacttgtttatttaaagacgggtctctttagcaaacctggagcttctccattcagatagctccgctgccattaaactccaggggttctcctgtctccacctttctgccaccgcagagctgggttagaagcccttgcccctgcaccggtctttaccatagactctggaatctaaactcagatcttcatgctcctgtggcagacactttacctactgaggcatctcctttgccctcggctgaggcacagcatgatttatccagagcagtcaggtctgtcccgtccatgatctccaagccttctgagcatccacaaccctggtgattagctagacacatcaagagacatcgtggatactgcccaagagaccagtgccccattcaagctcagacagtgaagttccagatccccatgagaagtggcctgacccctcatctgcccatctgcatgccctctgcaatctgttggctctgagtggcacagcttgctctgccctgccaagtggcaggagcttccattccaggagctggcaggagacacctgaagccggacagggctttatctcggagctggtgctgctgaataatggattcagcatgcgttcctgggctcctgcacacactcactcacacacacacacacacacacacacacacacacacacacacgcgcgctacacacatgctgggctgacaacccagaggggcggggctgccggggctgcacagctctgatgagctgaaggagcagcttgctttggttgccttggtctctgtgggcagcagcaggaggaggcggcagcagccagagaagagggaggcgtgtgagccacactccaccagcgagcttcttcccgctgctctggaactgccctttctttctctctttcttt

SEQ ID NO: 12 - DNA, 542 bp, SHH mini promoter; identical to SEQ ID NO: 7
  source 1..542: mol_type = other DNA

SEQ ID NO: 13 - DNA, 41 bp, upstream primer of otof promoter
  source 1..41: mol_type = other DNA
cacgcgttctcgattctagagtactacagcccacagaagag

SEQ ID NO: 14 - DNA, 43 bp, downstream primer of otof promoter
  source 1..43: mol_type = other DNA
cttcccgctgctctggaactgccctttctttctctctttcttt

SEQ ID NO: 15 - DNA, 20 bp, downstream homologous arm of otof
  source 1..20: mol_type = other DNA
gctagcgaattcgccaccat

SEQ ID NO: 16 - DNA, 339 bp, promoter Sox10
  source 1..339: mol_type = other DNA
cacgcgttctcgattctagagtggcctcaggcccctgtgcccgcgcccatggggttaaatctctccctgtctctctctgctccaagttgttttccaagcgaggcagagaatggttctcttgttaccaacatggcttctgggcattgggtaatgcgttccctcttctccctgccctgcgccacaaagggaccttttgttcctctcccggcccctctctctggctcttctctgccccccacccaccccaagtccctcctccccacgcctcctgccctactctgcgcgcacccctgggctgtgaggagtgaccgtggcctggctttctttctctctttcttt

SEQ ID NO: 17 - DNA, 542 bp, SHH mini promoter; identical to SEQ ID NO: 7
  source 1..542: mol_type = other DNA

SEQ ID NO: 18 - DNA, 20 bp, upstream homologous arm of Sox10
  source 1..20: mol_type = other DNA
cacgcgttctcgattctaga

SEQ ID NO: 19 - DNA, 20 bp, downstream homologous arm of Sox10
  source 1..20: mol_type = other DNA
ctttctttctctctttcttt

SEQ ID NO: 20 - DNA, 20 bp, downstream homologous arm
  source 1..20: mol_type = other DNA
gctagcgaattcgccaccat

SEQ ID NO: 21 - DNA, 940 bp, promoter Ngfr 1
  source 1..940: mol_type = other DNA
cacgcgttctcgattctagagatccgaagcatcttatgctcagcataaccggaggtgccctgggtacgtggggcagcccactgagaagccacagcggggcacacgggtgcggctcctctcacgcctcacttgactgctctggactccccaccctaggcagccgggcgggcgcggttccggaggggttgggggggggggggagttgggcgggctgggcggggaggaggcggggctgctgcattgccttcacccagctgctcccgcccgctagcagccagagcgagtggagcctccgccagctccggcgggcagcgggcgctggagcgcagcgcagcgcagctcagctcagcgcgcagcaccatcggtccgcagagcggactgagctagaagctgagcgctgtcgcagactgggagcagtctcgagtggggtggagggaggtttgggaatctcgggcgcctgggttcttttgacgacagcgtgtgaattttgggatcccgaggggagttttctctttagcatcttagtccctggggagttgtagggcagagagaaggaagggaaagagatcggcactaaagatgtgaggggctagagacggaacaatgcgggaggcagctggagggactggaggcagaggggacccagtatggacaatggggaccggccagacaatgggggggaggggcatcgaaaggagcgattcgggatagagccggttctgtgttccgccgcggaccgagcctcttcctgcgccgctgcgagagttctgaaaccagagcgcaaccagagtctgctggccggccgcgccggtaatggaggcactttgtcattcagacgtctgtaaccggagccgcccggctggctaatgctcctaatagggatgcagcagcgtaggcaacaaatgggcagcatgagcgtcctttctttctctctttcttt

SEQ ID NO: 22 - DNA, 542 bp, SHH mini promoter; identical to SEQ ID NO: 7
  source 1..542: mol_type = other DNA

SEQ ID NO: 23 - DNA, 20 bp, upstream homologous arm of promoter Ngfr 1
  source 1..20: mol_type = other DNA
cacgcgttctcgattctaga

SEQ ID NO: 24 - DNA, 20 bp, downstream homologous arm of promoter Ngfr 1
  source 1..20: mol_type = other DNA
ctttctttctctctttcttt

SEQ ID NO: 25 - DNA, 20 bp, downstream homologous arm
  source 1..20: mol_type = other DNA
gctagcgaattcgccaccat

SEQ ID NO: 26 - DNA, 1499 bp, Ngfr 2 promoter
  source 1..1499: mol_type = other DNA
cacgcgttctcgattctagagccgagctctatgtgatgaaaggaaatcagaacagacccttctgaaatctcagctcctgggagaagcctgcctcaagtacctcagggctcctggtctgcagatgttgccattgccagccagcactcccactgccagcacctgggaggagatggtggcagcttccggtgctgcctggactctctctgctgcccttatggagaccactctgcccctagggcatcacccagtgttttctcctgcctctgtttacttttctgtcaaactctggtgaaaccacagtggtgtgtgtgtgtgtgtgtgtgtgtgtgtgtgtgtggtgtgtcttggcaaagatcggtccagcatggaagcaggagaggaatgcccaaacaatcttgtaaagctctctggtctcacgaccaaagcccaaattgctcagcatcaaatggggtgggtggggggtgtgtgcgcaaggtctggagcctgcagagaaggctttggagttttattagacattaagattgttctttaaggaacagaaacaaagtgagcctccaacagcccctccctcgggggaatctggtgctaagtcgttccatccatgagcaaagatgctttagtggcaggaatctgactccccccccccccatccagctctgttcccaggggccacatgggaggagaggggaggggatggagtcaggctaggacggggaagtcaactctggaagaatagagttgctggctggtgaaagccggccactgataacaggcgtccctttctctgtcttggctccagacttgcccatcagtctttgccctggcaccaagctgtccctgtgtttatctgcagaggggtgaaaactcccaaaggaaacccagggcaggccagacacctccagtacagagtcaatatttgaacccaagtcctcactgccttctgttcttggacatagacaactccgttttgatatttaatatgtggaatgagacctggagaagggccctgttctcctttttaggaaagggccctgcctctgggtaactgcagccctgcaggtgtgaagtttagcaaatggagtttgggccaaatttcagttccactggcccccttggctaggagccctgtgcaagctgcaacctgcccagccattctggatatcggtctcaccctcctcctgtggtgtatcctcaggactccaggagaggctgtaaccctaaggtgaactctgcagaaggttagccactgaggctatgacctcacaccccagcagcagtcaagggccccactccccccacgccccccactgccccccagccttccttcctgccagctttgatcctcctaatgcctcccgggtgagctcatcccagcccaggtggttctaatagaaagtattaagagggaggcgtttgatcccttggaagacaccacctttgctcctgccaggctgaccttgtgatctccttccacctaggctttctttctctctttcttt

SEQ ID NO: 27 - DNA, 542 bp, SHH mini promoter; identical to SEQ ID NO: 7
  source 1..542: mol_type = other DNA

SEQ ID NO: 28 - DNA, 20 bp, upstream homologous arm of promoter Ngfr 2
  source 1..20: mol_type = other DNA
cacgcgttctcgattctaga

SEQ ID NO: 29 - DNA, 20 bp, downstream homologous arm of Ngfr 2
  source 1..20: mol_type = other DNA
ctttctttctctctttcttt

SEQ ID NO: 30 - DNA, 20 bp, downstream homologous arm
  source 1..20: mol_type = other DNA
gctagcgaattcgccaccat

SEQ ID NO: 31 - DNA, 2014 bp, Dnah5 promoter
  source 1..2014: mol_type = other DNA
gtcacatgttgacaatgttctcgggactaatctgaactgcttagcagggacgatcagactatcttgtcttattctgtgtctctcctgtgacctgtggccaccgttcacaattataacaacaaacagctgcttaccaatacacagaggttgattgaaaattatctttatatctcacgtatagtgtgcgcttcatttgcctgaggctctatgttaagtctgccgtgaccccggatgtattcacacaccatgttggctcagaagatgacactcccaaatgtacagctgtgaagtttagagtgagaacccgtgaagagccgcacattcagggagagttttctttctccttatctatcttcaagtccacatagtccaggagacattatttgctgcaagtgctttcctcagccatcccagcaggaagaggaaacacatgcaaatggcaggcaggagtgatggctaccacaggggcattaccccaaggcattgtctgttctttgagtcaattcatctccgtgaaaaataatctactcttccgataaaattgctcaatacttttttttctctcctcaaagaagaacagatgtaagcttctaaatcttactgaactgctgggcacctgggtgattcccgtgtgtgcaatactctgcatggcttctcccttgtcaatctgtctactgcctttgtcagattcaaacactgaacttccaagggaaaatagagagttcttctgtgcctatacttctgactttaaatatgcttttgttatttgcttgccatcagtattcaacaccaaatatctgtatccatattaacactacaaatggaggccacaccctaactggctgatggctaggtgaattgattgtcctgatatcaaggtagtgccctggttgtcaattctgtttctgatgaggttgaatagcaggggactcctcaatttcctgatgatctttgaataatccgaaaaggatttatttactagattttattttacgttttaatttttttgagatagagtttctctatgtagctgtagccatctggaactcctctgtaaaccaggctagcctggaactcacagatatcggcctctatctcctgagtgctgggattaaaggtgagcaccactgctgcctagctaactgctggatttttaatcccaaggatccaatgaaatggaccttaaattctgccatttgtgtgctttgatgggagggttgtaggtgagaggtctctccccatccgtcggtgcggagaggaagatctagatgtttaggcttatggaatgcaatgctttgctttccatgcttgggcggccgtgtgaacaggagtaatttatggacaccatttgccatttgcatatgaaataggctgcttgttctttatgggagaggaaatggctcctttgggtcacaattagcctatcaagcaattagtcacaattagtcaccatgctggcagttaattgtgcacacaaagttgtttagacaaagtaagactgaatttcctaactcgagtaatatatccagagctgtgacttgtctgccttctgctttgatcaggtttaaggtttcttattgttcagagaaataatttaagctcctttattgactcaaagcttattgttgggcagtgtatggaatggaacattagaacttgtggttgcaaccaagcagttaaattgctttctcttgttgctaaacatgattaagaggcgtgcttaaacggcacagcatggaaacagtattaccctaacaacgaaggaccacagaatcgaggaaaggccccagggcagagactcagggaaggatatatgagcatcgcagatggactgacttctcgcctcagttctgtgaatatcgagagtcacccacatgcatgagaagcaacagcgcgatgctgtgaccctcttagagtctttgcctgtgatattccactggaggatgaacagctctcttggtagttagaagaccattctggaggagctgacttggggccatcccagattgctggg

SEQ ID NO: 32 - DNA, 409 bp, CMV enhancer; identical to SEQ ID NO: 5
  source 1..409: mol_type = other DNA

SEQ ID NO: 33 - DNA, 44 bp, forward primer of primer pair G
  source 1..44: mol_type = other DNA
ctattaccatggtgctcgaggtcacatgttgacaatgttctcgg

SEQ ID NO: 34 - DNA, 39 bp, reverse primer of primer pair G
  source 1..39: mol_type = other DNA
gccatcccagattgctgggggtacctcgacggtaagtcc

SEQ ID NO: 35 - DNA, 24 bp, P1
  source 1..24: mol_type = other DNA
gagattatggcccttcagagtcac

SEQ ID NO: 36 - DNA, 24 bp, P2
  source 1..24: mol_type = other DNA
gagttgcagagcccagaggttagg

SEQ ID NO: 37 - DNA, 24 bp, P3
  source 1..24: mol_type = other DNA
gctgcttccttgatgcctcctaca

SEQ ID NO: 38 - DNA, 24 bp, P4
  source 1..24: mol_type = other DNA
tgctcaatggctgctcctcacttc